European Patent Specification EP 3 399 033 B1, published November 6, 2024. Title: Peptide tag and tagged protein comprising the same. Applicant: Idemitsu Kosan Co., Ltd. The sequence listing filed with the application follows.

SEQUENCE LISTING (186 sequences)

SEQ ID NO: 1 - protein, 191 aa, Homo sapiens
FPTIPLSRLFDNAMLRAHRLHQLAFDTYQEFEEAYIPKEQKYSFLQNPQTSLCFSESIPTPSNREETQQKSNLELLRISLLLIQSWLEPVQFLRSVFANSLVYGASDSNVYDLLKDLEEGIQTLMGRLEDGSPRIGQIFKQTYSKFDTNSHNDDALLKNYGLLYCFRKDMDKVETFLRIVQCRSVEGSCGF

SEQ ID NO: 2 - protein, 165 aa, Homo sapiens
SYNLLGFLQRSSNFQSQKLLWQLNGRLEYCLKDRMNFDIPEEIKQLQQFQKEDAALTIYEMLQNIFAIFRQDSSSTGWNETIVENLLANVYHQINHLKTVLEEKLEKEDFTRGKLMSSLHLKRYYGRILHYLKAKEYSHCAWTIVRVEILRNFYFINRLTGYLRN

SEQ ID NO: 3 - DNA, 573 bp, Homo sapiens
ttcccaaccattcccttatccaggctttttgacaacgctatgctccgcgcccatcgtctgcaccagctggcctttgacacctaccaggagtttgaagaagcctatatcccaaaggaacagaagtattcattcctgcagaacccccagacctccctctgtttctcagagtctattccgacaccctccaacagggaggaaacacaacagaaatccaacctagagctgctccgcatctccctgctgctcatccagtcgtggctggagcccgtgcagttcctcaggagtgtcttcgccaacagcctggtgtacggcgcctctgacagcaacgtctatgacctcctaaaggacctagaggaaggcatccaaacgctgatggggaggctggaagatggcagcccccggatcgggcagatcttcaagcagacctacagcaagttcgacacaaactcacacaacgatgacgcactactcaagaactacgggctgctctactgcttcaggaaggacatggacaaggtcgagacattcctgcgcatcgtgcagtgccgctctgtggagggcagctgtggcttc

SEQ ID NO: 4 - DNA, 495 bp, Homo sapiens
agctacaacttgcttggattcctacaaagaagcagcaattttcagtctcagaagctcctgtggcaattgaatgggaggcttgaatactgcctcaaggacaggatgaactttgacatccctgaggagattaagcagctgcagcagttccagaaggaggacgccgcattgaccatctatgagatgctccagaacatctttgctattttcagacaagattcatctagcactggctggaatgagactattgttgagaacctcctggctaatgtctatcatcagataaaccatctgaagacagtcctggaagaaaaactggagaaagaagatttcaccaggggaaaactcatgagcagtctgcacctgaaaagatattatgggaggattctgcattacctgaaggccaaggagtacagtcactgtgcctggaccatagtcagagtggaaatcctaaggaacttttacttcattaacagacttacaggttacctccgaaac

SEQ ID NO: 5 - protein, 19 aa, Saccharomyces cerevisiae
MLLQAFLFLLAGFAAKISA

SEQ ID NO: 6 - protein, 12 aa, Artificial Sequence
  HN tag
HNHNHNHNHNHN

SEQ ID NO: 7 - DNA, 137 bp, Artificial Sequence
  SUC2SP-6xHN-cloning site
atgcttttgcaagccttccttttcctcttggctggtttcgccgccaagatttctgcccataatcataatcataatcataatcataatcataatggcggccgcgtcgacggccagggtggccctcgagggcgcgccaa

SEQ ID NO: 8 - DNA, 41 bp, Artificial Sequence
  6XHN-hGHF
ataatcataatggcggccgcttcccaaccattcccttatcc

SEQ ID NO: 9 - DNA, 47 bp, Artificial Sequence
  hGHR-stopCYCt
gatgcggccctctagattggcgcgcctcagaagccacagctgccctc

SEQ ID NO: 10 - protein, 4 aa, Artificial Sequence
  FXa recognition sequence
IEGR

SEQ ID NO: 11 - DNA, 50 bp, Artificial Sequence
  6XHN-RS-hGHF
atcataatcataatggcggccgcagatccttcccaaccattcccttatcc

SEQ ID NO: 12 - protein, 12 aa, Artificial Sequence
  ECM29SC
RSPESGAGSPRS

SEQ ID NO: 13 - DNA, 86 bp, Artificial Sequence
  6XHN-ECM29SC-hGHF
atcataatcataatggcggccgcttgggttctgaatctgatgattctgaaggttctattaaacaattcccaaccattcccttatcc

SEQ ID NO: 14 - protein, 14 aa, Artificial Sequence
  ECM29ON
LGSESDDSEGSIKQ

SEQ ID NO: 15 - DNA, 80 bp, Artificial Sequence
  6XHN-ECM29ON-hGHF
atcataatcataatggcggccgcagatcccctgaatctggtgctggttctcctagatccttcccaaccattcccttatcc

SEQ ID NO: 16 - protein, 14 aa, Artificial Sequence
  Anjam-N
GPGPSRGSDIKLTS

SEQ ID NO: 17 - DNA, 86 bp, Artificial Sequence
  6XHN-Anjam-hGHF
atcataatcataatggcggccgcggtcctggtccttctagaggttctgatattaaattgacttctttcccaaccattcccttatcc

SEQ ID NO: 18 - protein, 12 aa, Artificial Sequence
  PG12v5
RWPGSGPGWPRS

SEQ ID NO: 19 - DNA, 80 bp, Artificial Sequence
  6XHN-PG12v5-hGHF
atcataatcataatggcggccgcagatggcctggtttgggtcctggttggcctacttccttcccaaccattcccttatcc

SEQ ID NO: 20 - protein, 12 aa, Artificial Sequence
  PG12v7
PSGPSGPGSPTS

SEQ ID NO: 21 - DNA, 80 bp, Artificial Sequence
  6XHN-PG12v7-hGHF
atcataatcataatggcggccgcccttccggtccttctggtcctggttctcctacttccttcccaaccattcccttatcc

SEQ ID NO: 22 - protein, 12 aa, Artificial Sequence
  PG12
RSPGSGPGSPRS

SEQ ID NO: 23 - DNA, 80 bp, Artificial Sequence
  6XHN-PG12-hGHF
atcataatcataatggcggccgcagatcccctggttctggtcctggttctcctagatccttcccaaccattcccttatcc

SEQ ID NO: 24 - DNA, 78 bp, Artificial Sequence
  hGHR-PG12-stopCYCt
ggccctctagattggcgcgcctcaggatctaggagaaccaggaccagaaccaggggatctgaagccacagctgccctc

SEQ ID NO: 25 - protein, 12 aa, Artificial Sequence
  PX12-20
RKPGKGPGKPRS

SEQ ID NO: 26 - DNA, 80 bp, Artificial Sequence
  6XHN-PX12-20-hGHF
atcataatcataatggcggccgcagaaaacctggtaaaggtcctggtaaacctagatccttcccaaccattcccttatcc

SEQ ID NO: 27 - DNA, 80 bp, Artificial Sequence
  hGHR-PX12-20-stopCYCt
gcggccctctagattggcgcgcctcaggatctaggtttaccaggacctttaccaggttttctgaagccacagctgccctc

SEQ ID NO: 28 - protein, 12 aa, Artificial Sequence
  PX12-20v2
RKPGKGPGKPRK

SEQ ID NO: 29 - DNA, 77 bp, Artificial Sequence
  6XHN-PX12-20v2-hGHF
ataatcataatggcggccgcagaaaacctggtaaaggtcctggtaaacctagaaaattcccaaccattcccttatcc

SEQ ID NO: 30 - protein, 12 aa, Artificial Sequence
  PX12-20v3
RKPGKGPGKPTS

SEQ ID NO: 31 - DNA, 77 bp, Artificial Sequence
  6XHN-PX12-20v3-hGHF
ataatcataatggcggccgcagaaaacctggtaaaggtcctggtaaacctacttccttcccaaccattcccttatcc

SEQ ID NO: 32 - protein, 12 aa, Artificial Sequence
  PX12-20v4
RKPGKGPGKPLS

SEQ ID NO: 33 - DNA, 77 bp, Artificial Sequence
  6XHN-PX12-20v4-hGHF
ataatcataatggcggccgcagaaaacctggtaaaggtcctggtaaacctttgtccttcccaaccattcccttatcc

SEQ ID NO: 34 - protein, 12 aa, Artificial Sequence
  PX12-20v5
TKPGKGPGKPTS

SEQ ID NO: 35 - DNA, 77 bp, Artificial Sequence
  6XHN-PX12-20v5-hGHF
ataatcataatggcggccgcactaaacctggtaaaggtcctggtaaacctacttccttcccaaccattcccttatcc

SEQ ID NO: 36 - protein, 12 aa, Artificial Sequence
  PX12-20v6
KKPGKGPGKPKK

SEQ ID NO: 37 - DNA, 77 bp, Artificial Sequence
  6XHN-PX12-20v6-hGHF
ataatcataatggcggccgcaaaaaacctggtaaaggtcctggtaaacctaaaaaattcccaaccattcccttatcc

SEQ ID NO: 38 - protein, 12 aa, Artificial Sequence
  PX12-20v7
RKPKKKPKKPRS

SEQ ID NO: 39 - DNA, 77 bp, Artificial Sequence
  6XHN-PX12-20v7-hGHF
ataatcataatggcggccgcagaaaacctaaaaaaaaacctaaaaaacctagatccttcccaaccattcccttatcc

SEQ ID NO: 40 - protein, 12 aa, Artificial Sequence
  PX12-20v8
RKPGKGPGSPRS

SEQ ID NO: 41 - DNA, 77 bp, Artificial Sequence
  6XHN-PX12-20v8-hGHF
ataatcataatggcggccgcagatcccctggtaaaggtcctggtaaacctagatccttcccaaccattcccttatcc

SEQ ID NO: 42 - protein, 12 aa, Artificial Sequence
  PX12-20v9
RKPGSGPGKPRS

SEQ ID NO: 43 - DNA, 77 bp, Artificial Sequence
  6XHN-PX12-20v9-hGHF
ataatcataatggcggccgcagaaaacctggttctggtcctggtaaacctagatccttcccaaccattcccttatcc

SEQ ID NO: 44 - protein, 12 aa, Artificial Sequence
  PX12-29
RKPGKPKGKPTS

SEQ ID NO: 45 - DNA, 77 bp, Artificial Sequence
  6XHN-PX12-29-hGHF
ataatcataatggcggccgcagaaaacctggtaaacctaaaggtaaacctacttccttcccaaccattcccttatcc

SEQ ID NO: 46 - protein, 12 aa, Artificial Sequence
  PX12-32
RQPGQGPGQPRS

SEQ ID NO: 47 - DNA, 77 bp, Artificial Sequence
  6XHN-PX12-32-hGHF
ataatcataatggcggccgcagacaacctggtcaaggtcctggtcaacctagatccttcccaaccattcccttatcc

SEQ ID NO: 48 - protein, 12 aa, Artificial Sequence
  PX12-33
RNPGNGPGNPRS

SEQ ID NO: 49 - DNA, 77 bp, Artificial Sequence
  6XHN-PX12-33-hGHF
ataatcataatggcggccgcagaaatcctggtaatggtcctggtaatcctagatccttcccaaccattcccttatcc

SEQ ID NO: 50 - protein, 12 aa, Artificial Sequence
  PX12-36
RLPGLGPGLPRS

SEQ ID NO: 51 - DNA, 77 bp, Artificial Sequence
  6XHN-PX12-36-hGHF
ataatcataatggcggccgcagattgcctggtttgggtcctggtttgcctagatccttcccaaccattcccttatcc

SEQ ID NO: 52 - protein, 12 aa, Artificial Sequence
  PX12-38
RRPGRGPGRPRS

SEQ ID NO: 53 - DNA, 77 bp, Artificial Sequence
  6XHN-PX12-38-hGHF
ataatcataatggcggccgcagaagacctggtagaggtcctggtagacctagatccttcccaaccattcccttatcc

SEQ ID NO: 54 - protein, 12 aa, Artificial Sequence
  PX12-28
RSPKSKPKSPRS

SEQ ID NO: 55 - DNA, 77 bp, Artificial Sequence
  6XHN-PX12-28-hGHF
ataatcataatggcggccgcagatcccctaaatctaaacctaaatctcctagatccttcccaaccattcccttatcc

SEQ ID NO: 56 - protein, 12 aa, Artificial Sequence
  PX12-39
RSPGSGPGSPTS

SEQ ID NO: 57 - DNA, 77 bp, Artificial Sequence
  6XHN-PX12-39-hGHF
ataatcataatggcggccgcagatcccctggttctggtcctggttctcctacttccttcccaaccattcccttatcc

SEQ ID NO: 58 - protein, 17 aa, Artificial Sequence
  PX17-20
RKPGKGPGKPRKPGKRS

SEQ ID NO: 59 - DNA, 92 bp, Artificial Sequence
  6XHN-PX17-20-hGHF
ataatcataatggcggccgcagaaaacctggtaaaggtcctggtaaacctagaaaacctggtaaaagatccttcccaaccattcccttatcc

SEQ ID NO: 60 - protein, 17 aa, Artificial Sequence
  PX17-20v2
RKPGKGPGKPRSPGSRS

SEQ ID NO: 61 - DNA, 92 bp, Artificial Sequence
  6XHN-PX17-20v2-hGHF
ataatcataatggcggccgcagaaaacctggtaaaggtcctggtaaacctagatcccctggttctagatccttcccaaccattcccttatcc

SEQ ID NO: 62 - protein, 16 aa, Artificial Sequence
  PX12-20Xa
RKPGKGPGKPRSIEGR

SEQ ID NO: 63 - DNA, 89 bp, Artificial Sequence
  6XHN-PX12-20Xa-hGHF
ataatcataatggcggccgcagaaaacctggtaaaggtcctggtaaacctagatccattgaaggtagattcccaaccattcccttatcc

SEQ ID NO: 64 - protein, 11 aa, Artificial Sequence
  PK11v1
RKPGKGPGKPR

SEQ ID NO: 65 - DNA, 74 bp, Artificial Sequence
  6XHN-PK11v1-hGHF
ataatcataatggcggccgcagaaaacctggtaaaggtcctggtaaacctagattcccaaccattcccttatcc

SEQ ID NO: 66 - protein, 11 aa, Artificial Sequence
  PK11v2
KPGKGPGKPRS

SEQ ID NO: 67 - DNA, 74 bp, Artificial Sequence
  6XHN-PK11v2-hGHF
ataatcataatggcggccgcaaacctggtaaaggtcctggtaaacctagatccttcccaaccattcccttatcc

SEQ ID NO: 68 - DNA, 41 bp, Artificial Sequence
  6XHN-IFNBF
ataatcataatggcggccgcagctacaacttgcttggattc

SEQ ID NO: 69 - DNA, 52 bp, Artificial Sequence
  IFNBR-stopCYCt
gatgcggccctctagattggcgcgcctcagtttcggaggtaacctgtaagtc

SEQ ID NO: 70 - DNA, 77 bp, Artificial Sequence
  6XHN-PG12-IFNBF
ataatcataatggcggccgcagatcccctggttctggtcctggttctcctagatccagctacaacttgcttggattc

SEQ ID NO: 71 - DNA, 80 bp, Artificial Sequence
  IFNBR-PG12-stopCYCt
ggccctctagattggcgcgcctcaggatctaggagaaccaggaccagaaccaggggatctgtttcggaggtaacctgtaa

SEQ ID NO: 72 - DNA, 77 bp, Artificial Sequence
  6XHN-PX12-20-IFNBF
ataatcataatggcggccgcagaaaacctggtaaaggtcctggtaaacctagatccagctacaacttgcttggattc

SEQ ID NO: 73 - DNA, 80 bp, Artificial Sequence
  IFNBR-PX12-20-stopCYCt
ggccctctagattggcgcgcctcaggatctaggtttaccaggacctttaccaggttttctgtttcggaggtaacctgtaa

SEQ ID NO: 74 - DNA, 47 bp, Artificial Sequence
  hGHR-stopT7t
tttgttagcagccggatcggcgcgcctcagaagccacagctgccctc

SEQ ID NO: 75 - DNA, 80 bp, Artificial Sequence
  hGHR-PX12-20-stopT7t
gttagcagccggatcggcgcgcctcaggatctaggtttaccaggacctttaccaggttttctgaagccacagctgccctc

SEQ ID NO: 76 - DNA, 52 bp, Artificial Sequence
  IFNBR-stopT7t
tttgttagcagccggatcggcgcgcctcagtttcggaggtaacctgtaagtc

SEQ ID NO: 77 - DNA, 80 bp, Artificial Sequence
  IFNBR-PX12-20-stopT7t
tagcagccggatcggcgcgcctcaggatctaggtttaccaggacctttaccaggttttctgtttcggaggtaacctgtaa

SEQ ID NO: 78 - DNA, 231 bp, Artificial Sequence
  RBS-PelBSP-6xHN-cloning site-CYCt
aataattttgtttaactttaagaaggagatatacatatgaaatacctgctgccgaccgctgctgctggtctgctgctcctcgctgcccagccggcgatggcccataatcataatcataatcataatcataatcataatggcggccgcgtcgacggccagggtggccctcgagggcgcgccgatccggctgctaacaaagcccgaaaggaagctgagttggctgctgccacc

SEQ ID NO: 79 - DNA, 77 bp, Artificial Sequence
  6XHN-PX12-62-hGHF
ataatcataatggcggccgcagaaatcctaaaaataaacctaaaaatcctagatccttcccaaccattcccttatcc

SEQ ID NO: 80 - DNA, 80 bp, Artificial Sequence
  hGHR-PX12-20v7-stopT7t
gttagcagccggatcggcgcgcctcaggatctaggttttttaggtttttttttaggttttctgaagccacagctgccctc

SEQ ID NO: 81 - DNA, 77 bp, Artificial Sequence
  6XHN-PX12-20v7-IFNBF
ataatcataatggcggccgcagaaaacctaaaaaaaaacctaaaaaacctagatccagctacaacttgcttggattc

SEQ ID NO: 82 - DNA, 80 bp, Artificial Sequence
  IFNBR-PX12-20v7-stopT7t
tagcagccggatcggcgcgcctcaggatctaggttttttaggtttttttttaggttttctgtttcggaggtaacctgtaa

SEQ ID NO: 83 - DNA, 43 bp, Artificial Sequence
  P22SP-hGHF
agtaccaagttccgcattcgctttcccaaccattcccttatcc

SEQ ID NO: 84 - DNA, 36 bp, Artificial Sequence
  hGHR-stopBrevit
catcctgttaagctttcagaagccacagctgccctc

SEQ ID NO: 85 - DNA, 72 bp, Artificial Sequence
  P22SP-PX12-20-hGHF
agttccgcattcgctagaaaacctggtaaaggtcctggtaaacctagatccttcccaaccattcccttatcc

SEQ ID NO: 86 - DNA, 72 bp, Artificial Sequence
  hGHR-PX12-20-stopBrevit
catcctgttaagctttcaggatctaggtttaccaggacctttaccaggttttctgaagccacagctgccctc

SEQ ID NO: 87 - DNA, 72 bp, Artificial Sequence
  P22SP-PX12-38-hGHF
agttccgcattcgctagaagacctggtagaggtcctggtagacctagatccttcccaaccattcccttatcc

SEQ ID NO: 88 - DNA, 72 bp, Artificial Sequence
  hGHR-PX12-38-stopBrevit
catcctgttaagctttcaggatctaggtctaccaggacctctaccaggtcttctgaagccacagctgccctc

SEQ ID NO: 89 - DNA, 72 bp, Artificial Sequence
  P22SP-PX12-20v7-hGHF
agttccgcattcgctagaaaacctaaaaaaaaacctaaaaaacctagatccttcccaaccattcccttatcc

SEQ ID NO: 90 - DNA, 72 bp, Artificial Sequence
  hGHR-PX12-20v7-stopBrevit
catcctgttaagctttcaggatctaggttttttaggtttttttttaggttttctgaagccacagctgccctc

SEQ ID NO: 91 - DNA, 80 bp, Artificial Sequence
  hGHR-PX12-20v7-stopCYCt
gcggccctctagattggcgcgcctcaggatctaggttttttaggtttttttttaggttttctgaagccacagctgccctc

SEQ ID NO: 92 - protein, 12 aa, Artificial Sequence
  PX12-40
RRPRRRPRRPRS

SEQ ID NO: 93 - DNA, 77 bp, Artificial Sequence
  6XHN-PX12-40-hGHF
ataatcataatggcggccgcagaagacctagaagaagacctagaagacctagatccttcccaaccattcccttatcc

SEQ ID NO: 94 - protein, 12 aa, Artificial Sequence
  PX12-41
RRPKRKPKRPRS

SEQ ID NO: 95 - DNA, 77 bp, Artificial Sequence
  6XHN-PX12-41-hGHF
ataatcataatggcggccgcagaagacctaaaagaaaacctaaaagacctagatccttcccaaccattcccttatcc

SEQ ID NO: 96 - protein, 12 aa, Artificial Sequence
  PX12-43
RKPRKRPRKPRS

SEQ ID NO: 97 - DNA, 77 bp, Artificial Sequence
  6XHN-PX12-43-hGHF
ataatcataatggcggccgcagaaaacctagaaaaagacctagaaaacctagatccttcccaaccattcccttatcc

SEQ ID NO: 98 - protein, 12 aa, Artificial Sequence
  PX12-44
KKPKKKPKKPKK

SEQ ID NO: 99 - DNA, 77 bp, Artificial Sequence
  6XHN-PX12-44-hGHF
ataatcataatggcggccgcaaaaaacctaaaaaaaaacctaaaaaacctaaaaaattcccaaccattcccttatcc

SEQ ID NO: 100 - protein, 17 aa, Artificial Sequence
  PX17-20v7
RKPKKKPKKPRKPKKRS

SEQ ID NO: 101 - DNA, 92 bp, Artificial Sequence
  6XHN-PX17-20v7-hGHF
ataatcataatggcggccgcagaaaacctaaaaaaaaacctaaaaaacctagaaaacctaaaaaaagatccttcccaaccattcccttatcc

SEQ ID NO: 102 - protein, 17 aa, Artificial Sequence
  PX17-20v8
RKPKKKPKKPKKPKKRS

SEQ ID NO: 103 - DNA, 92 bp, Artificial Sequence
  6XHN-PX17-20v8-hGHF
ataatcataatggcggccgcagaaaacctaaaaaaaaacctaaaaaacctaaaaaacctaaaaaaagatccttcccaaccattcccttatcc

SEQ ID NO: 104 - protein, 13 aa, Artificial Sequence
  PX13-01
RKPKKKPKKKPRS

SEQ ID NO: 105 - DNA, 80 bp, Artificial Sequence
  6XHN-PX13-01-hGHF
ataatcataatggcggccgcagaaaacctaaaaaaaaacctaaaaaaaaacctagatccttcccaaccattcccttatcc

SEQ ID NO: 106 - protein, 12 aa, Artificial Sequence
  PX12-45
RKPKKPKKPKRS

SEQ ID NO: 107 - DNA, 77 bp, Artificial Sequence
  6XHN-PX12-45-hGHF
ataatcataatggcggccgcagaaaacctaaaaaacctaaaaaacctaaaagatccttcccaaccattcccttatcc

SEQ ID NO: 108 - protein, 22 aa, Artificial Sequence
  PX22-20v7
RKPKKKPKKPRKPKKKPKKPRS

SEQ ID NO: 109 - DNA, 107 bp, Artificial Sequence
  6XHN-PX22-20v7-hGHF
ataatcataatggcggccgcagaaaacctaaaaaaaaacctaaaaaacctagaaaacctaaaaaaaaacctaaaaaacctagatccttcccaaccattcccttatcc

SEQ ID NO: 110 - protein, 32 aa, Artificial Sequence
  PX32-20v7
RKPKKKPKKPRKPKKKPKKPRKPKKKPKKPRS

SEQ ID NO: 111 - DNA, 137 bp, Artificial Sequence
  6XHN-PX32-20v7-hGHF
ataatcataatggcggccgcagaaaacctaaaaaaaaacctaaaaaacctagaaaacctaaaaaaaaacctaaaaaacctagaaaacctaaaaaaaaacctaaaaaacctagatccttcccaaccattcccttatcc

SEQ ID NO: 112 - protein, 12 aa, Artificial Sequence
  PX12-20v9
RKPKSKPKKPRS

SEQ ID NO: 113 - DNA, 77 bp, Artificial Sequence
  6XHN-PX12-20v9-hGHF
ataatcataatggcggccgcagaaaacctaaatctaaacctaaaaaacctagatccttcccaaccattcccttatcc

SEQ ID NO: 114 - protein, 12 aa, Artificial Sequence
  PX12-20v10
RKPKGKPKKPRS

SEQ ID NO: 115 - DNA, 77 bp, Artificial Sequence
  6XHN-PX12-20v10-hGHF
ataatcataatggcggccgcagaaaacctaaaggtaaacctaaaaaacctagatccttcccaaccattcccttatcc

SEQ ID NO: 116 - protein, 12 aa, Artificial Sequence
  PX12-20v12
RKPGKKPGKPRS

SEQ ID NO: 117 - DNA, 77 bp, Artificial Sequence
  6XHN-PX12-20v12-hGHF
ataatcataatggcggccgcagaaaacctggtaaaaaacctggtaaacctagatccttcccaaccattcccttatcc

SEQ ID NO: 118 - protein, 12 aa, Artificial Sequence
  PX12-20v13
RKPGGKPGKPRS

SEQ ID NO: 119 - DNA, 77 bp, Artificial Sequence
  6XHN-PX12-20v13-hGHF
ataatcataatggcggccgcagaaaacctggtggtaaacctggtaaacctagatccttcccaaccattcccttatcc

SEQ ID NO: 120 - protein, 10 aa, Artificial Sequence
  PK10v2
RKPKKKPRKP

SEQ ID NO: 121 - DNA, 71 bp, Artificial Sequence
  6XHN-PK10v2-hGHF
ataatcataatggcggccgcagaaaacctaaaaaaaaacctagaaaacctttcccaaccattcccttatcc

SEQ ID NO: 122 - protein, 9 aa, Artificial Sequence
  PK09v2
RKPKKKPRK

SEQ ID NO: 123 - DNA, 68 bp, Artificial Sequence
  6XHN-PK09v2-hGHF
ataatcataatggcggccgcagaaaacctaaaaaaaaacctagaaaattcccaaccattcccttatcc

SEQ ID NO: 124 - protein, 10 aa, Artificial Sequence
  PK10v3
RPKKKPKKPR

SEQ ID NO: 125 - DNA, 71 bp, Artificial Sequence
  6XHN-PK10v3-hGHF
ataatcataatggcggccgcagacctaaaaaaaaacctaaaaaacctagattcccaaccattcccttatcc

SEQ ID NO: 126 - protein, 8 aa, Artificial Sequence
  PK08v3
RPKRKPRK

SEQ ID NO: 127 - DNA, 65 bp, Artificial Sequence
  6XHN-PK08v3-hGHF
ataatcataatggcggccgcagacctaaaagaaaacctagaaaattcccaaccattcccttatcc

SEQ ID NO: 128 - protein, 9 aa, Artificial Sequence
  PK09v3
PRKPRKPRK

SEQ ID NO: 129 - DNA, 68 bp, Artificial Sequence
  6XHN-PK09v3-hGHF
ataatcataatggcggccgccctagaaaacctagaaaacctagaaaattcccaaccattcccttatcc

SEQ ID NO: 130 - protein, 9 aa, Artificial Sequence
  PK09v4
PKRPKRPKR

SEQ ID NO: 131 - DNA, 68 bp, Artificial Sequence
  6XHN-PK09v4-hGHF
ataatcataatggcggccgccctaaaagacctaaaagacctaaaagattcccaaccattcccttatcc

SEQ ID NO: 132 - protein, 12 aa, Artificial Sequence
  PX12-49
RKPKLKPKKPRS

SEQ ID NO: 133 - DNA, 77 bp, Artificial Sequence
  6XHN-PX12-49-hGHF
ataatcataatggcggccgcagaaaacctaaattgaaacctaaaaaacctagatccttcccaaccattcccttatcc

SEQ ID NO: 134 - protein, 12 aa, Artificial Sequence
  PX12-51
RRPLRLPLRPRS

SEQ ID NO: 135 - DNA, 77 bp, Artificial Sequence
  6XHN-PX12-51-hGHF
ataatcataatggcggccgcagaagacctttgagattgcctttgagacctagatccttcccaaccattcccttatcc

SEQ ID NO: 136 - protein, 12 aa, Artificial Sequence
  PX12-52
RQPKQKPKQPRS

SEQ ID NO: 137 - DNA, 77 bp, Artificial Sequence
  6XHN-PX12-52-hGHF
ataatcataatggcggccgcagacaacctaaacaaaaacctaaacaacctagatccttcccaaccattcccttatcc

SEQ ID NO: 138 - protein, 12 aa, Artificial Sequence
  PX12-54
RQPKKKPKQPRS

SEQ ID NO: 139 - DNA, 77 bp, Artificial Sequence
  6XHN-PX12-54-hGHF
ataatcataatggcggccgcagacaacctaaaaaaaaacctaaacaacctagatccttcccaaccattcccttatcc

SEQ ID NO: 140 - protein, 12 aa, Artificial Sequence
  PX12-61
RHPKHKPKHPRS

SEQ ID NO: 141 - DNA, 77 bp, Artificial Sequence
  6XHN-PX12-61-hGHF
ataatcataatggcggccgcagacatcctaaacataaacctaaacatcctagatccttcccaaccattcccttatcc

SEQ ID NO: 142 - protein, 12 aa, Artificial Sequence
  PX12-62
RNPKNKPKNPRS

SEQ ID NO: 143 - protein, 12 aa, Artificial Sequence
  PX12-40v2
RRPRRPRRPRRS

SEQ ID NO: 144 - DNA, 77 bp, Artificial Sequence
  primer 6XHN-PX12-40v2-hGHF
ataatcataatggcggccgcagaagacctagaagacctagaagacctagaagatccttcccaaccattcccttatcc

SEQ ID NO: 145 - protein, 12 aa, Artificial Sequence
  PX12-41v2
RRPKRPKRPKRS

SEQ ID NO: 146 - DNA, 77 bp, Artificial Sequence
  primer 6XHN-PX12-41v2-hGHF
ataatcataatggcggccgcagaagacctaaaagacctaaaagacctaaaagatccttcccaaccattcccttatcc

SEQ ID NO: 147 - protein, 11 aa, Artificial Sequence
  PX12-45v2
RKPKKPKKPRS

SEQ ID NO: 148 - DNA, 74 bp, Artificial Sequence
  primer 6XHN-PX12-45v2-hGHF
ataatcataatggcggccgcagaaaacctaaaaaacctaaaaaacctagatccttcccaaccattcccttatcc

SEQ ID NO: 149 - protein, 13 aa, Artificial Sequence
  PX12-45v3
RKPKKPKKPKKRS

SEQ ID NO: 150 - DNA, 80 bp, Artificial Sequence
  primer 6XHN-PX12-45v3-hGHF
ataatcataatggcggccgcagaaaacctaaaaaacctaaaaaacctaaaaaaagatccttcccaaccattcccttatcc

SEQ ID NO: 151 - protein, 12 aa, Artificial Sequence
  PX12-75
RKPGSKPGKPRS

SEQ ID NO: 152 - DNA, 77 bp, Artificial Sequence
  primer 6XHN-PX12-75-hGHF
ataatcataatggcggccgcagaaaacctggttctaaacctggtaaacctagatccttcccaaccattcccttatcc

SEQ ID NO: 153 - protein, 12 aa, Artificial Sequence
  PX12-76
RKPQQKPQKPRS

SEQ ID NO: 154 - DNA, 77 bp, Artificial Sequence
  primer 6XHN-PX12-76-hGHF
ataatcataatggcggccgcagaaaacctcaacaaaaacctcaaaaacctagatccttcccaaccattcccttatcc

SEQ ID NO: 155 - protein, 12 aa, Artificial Sequence
  PX12-77
RRPGSRPGRPRS

SEQ ID NO: 156 - DNA, 77 bp, Artificial Sequence
  primer 6XHN-PX12-77-hGHF
ataatcataatggcggccgcagaagacctggttctagacctggtagacctagatccttcccaaccattcccttatcc

SEQ ID NO: 157 - protein, 11 aa, Artificial Sequence
  PX12-78
RKPKPKPKPRS

SEQ ID NO: 158 - DNA, 74 bp, Artificial Sequence
  primer 6XHN-PX12-78-hGHF
ataatcataatggcggccgcagaaaacctaaacctaaacctaaacctagatccttcccaaccattcccttatcc

SEQ ID NO: 159 - protein, 185 aa, Bacillus subtilis
ASPDYWQNWTDGGGTVNAVNGPGGNYSVNWSNTGNFVVGKGWTTGSPSRTINYNAGVWAPNGNGYLALYGWTRSPLIEYYVVDSWGTYRPTGTYKGTVKSDGGTYDIYTTTRYNAPSIDGEKTTFTQYWSVRQTKRPTGSNAKITFSNHVRAWKSHGMNLGSIWSYQVLATEGYQSSGSSNVTVW

SEQ ID NO: 160 - DNA, 555 bp, Bacillus subtilis
gctagcccagactactggcaaaattggactgatggcggcggaacagtaaacgctgtcaatgggcctggagggaattacagtgttaattggtctaataccggaaatttcgttgttggtaaaggttggactacaggttcgccatctaggacaataaactataatgccggagtttgggcgccgaatggcaatggatatttggctttatatggttggacgagatcacctctcatagaatattatgtagtggattcatggggtacttatagacctactggaacgtataaaggtactgtaaaaagtgatggcggcacatatgacatatatacaactacacgttataatgcaccttccattgatggcgaaaaaactactttcacgcagtactggagtgttcgccagacgaagagaccaactggaagcaacgctaaaatcactttcagcaatcatgttagagcatggaagagtcatggaatgaatctgggtagtatttggtcttatcaagtcttagcgacagagggatatcaaagtagtggaagttctaacgtaacagtgtgg

SEQ ID NO: 161 - protein, 9 aa, Artificial Sequence
  HA
YPYDVPDYA

SEQ ID NO: 162 - protein, 6 aa, Artificial Sequence
  6XHis
HHHHHH

SEQ ID NO: 163 - DNA, 56 bp, Artificial Sequence
  primer HA-6XHis
ctttcgcttacccatatgatgtaccagattacgctcatcatcatcatcatcattga

SEQ ID NO: 164 - DNA, 54 bp, Artificial Sequence
  primer mCWSP-AD-BsxynAF
acttactgttgctcccatggctttcgctgcagatgctagcccagactactggca

SEQ ID NO: 165 - DNA, 44 bp, Artificial Sequence
  primer BsxynAR-HA
gtaatctggtacatcatatgggtaccacactgttacgttagaac

SEQ ID NO: 166 - DNA, 90 bp, Artificial Sequence
  primer mCWSP-AD-PX12-20-BsxynAF
acttactgttgctcccatggctttcgctgcagatagaaaacctggtaaaggtcctggtaaacctagatccgctagcccagactactggca

SEQ ID NO: 167 - DNA, 80 bp, Artificial Sequence
  primer BsxynAR-PX12-20-HA
gtaatctggtacatcatatgggtaggatctaggtttaccaggacctttaccaggttttctccacactgttacgttagaac

SEQ ID NO: 168 - protein, 89 aa, Saccharomyces cerevisiae
MRFPSIFTAVLFAASSALAAPVNTTTEDETAQIPAEAVIGYSDLEGDFDVAVLPFSNSTNNGLLFINTTIASIAAKEEGVSLEKREAEA

SEQ ID NO: 169 - DNA, 280 bp, Artificial Sequence
  kozak-AFSP-stop
gatccaaacgatgagatttccttcaatttttactgcagttttattcgcagcatcctccgcattagctgctccagtcaacactacaacagaagatgaaacggcacaaattccggctgaagctgtcatcggttactcagatttagaaggggatttcgatgttgctgttttgccattttccaacagcacaaataacgggttattgtttataaatactactattgccagcattgctgctaaagaagaaggggtatctctcgagaaaagagaggctgaagcttga

SEQ ID NO: 170 - DNA, 61 bp, Artificial Sequence
  AFSP-hGH
agaagaaggggtatctctcgagaaaagagaggctgaagctttcccaaccattcccttatcc

SEQ ID NO: 171 - DNA, 52 bp, Artificial Sequence
  hGHR-stopAOXt
attctgacatcctcttgagcggccgcccctcagaagccacagctgccctcca

SEQ ID NO: 172 - DNA, 97 bp, Artificial Sequence
  AFSP-PX12-20-hGH
agaagaaggggtatctctcgagaaaagagaggctgaagctagaaaacctggtaaaggtcctggtaaacctagatccttcccaaccattcccttatcc

SEQ ID NO: 173 - DNA, 88 bp, Artificial Sequence
  hGHextR-PX12-20-stopAOXt
attctgacatcctcttgagcggccgcccctcaggatctaggtttaccaggacctttaccaggttttctgaagccacagctgccctcca

SEQ ID NO: 174 - DNA, 97 bp, Artificial Sequence
  AFSP-PX12-20v7-hGH
agaagaaggggtatctctcgagaaaagagaggctgaagctagaaaacctaaaaaaaaacctaaaaaacctagatccttcccaaccattcccttatcc

SEQ ID NO: 175 - protein, 238 aa, Aequorea victoria
MSGGEELFAGIVPVLIELDGDVHGHKFSVRGEGEGDADYGKLEIKFICTTGKLPVPWPTLVTTLCYGIQCFARYPEHMKMNDFFKSAMPEGYIQERTIQFQDDGKYKTRGEVKFEGDTLVNRIELKGKDFKEDGNILGHKLEYSFNSHNVYIRPDKANNGLEANFKTRHNIEGGGVQLADHYQTNVPLGDGPVLIPINHYLSTQTKISKDRNEARDHMVLLESFSACCHTHGMDELYR

SEQ ID NO: 176 - DNA, 717 bp, Aequorea victoria
atgagcgggggcgaggagctgttcgccggcatcgtgcccgtgctgatcgagctggacggcgacgtgcacggccacaagttcagcgtgcgcggcgagggcgagggcgacgccgactacggcaagctggagatcaagttcatctgcaccaccggcaagctgcccgtgccctggcccaccctggtgaccaccctctgctacggcatccagtgcttcgcccgctaccccgagcacatgaagatgaacgacttcttcaagagcgccatgcccgagggctacatccaggagcgcaccatccagttccaggacgacggcaagtacaagacccgcggcgaggtgaagttcgagggcgacaccctggtgaaccgcatcgagctgaagggcaaggacttcaaggaggacggcaacatcctgggccacaagctggagtacagcttcaacagccacaacgtgtacatccgccccgacaaggccaacaacggcctggaggctaacttcaagacccgccacaacatcgagggcggcggcgtgcagctggccgaccactaccagaccaacgtgcccctgggcgacggccccgtgctgatccccatcaaccactacctgagcactcagaccaagatcagcaaggaccgcaacgaggcccgcgaccacatggtgctcctggagtccttcagcgcctgctgccacacccacggcatggacgagctgtacaggtaa

SEQ ID NO: 177 - DNA, 37 bp, Artificial Sequence
  primer pENTR1A-1
agtcgactggatccggtaccgccaccatgagcggggg

SEQ ID NO: 178 - DNA, 80 bp, Artificial Sequence
  primer pENTR1A-2
agtcgactggatccggtaccgccaccatgaggtcccccggctccggccccggctcccccaggtccagcgggggcgaggag

SEQ ID NO: 179 - DNA, 80 bp, Artificial Sequence
  primer pENTR1A-3
agtcgactggatccggtaccgccaccatgaggaagcccggcaagggccccggcaagcccaggtccagcgggggcgaggag

SEQ ID NO: 180 - DNA, 80 bp, Artificial Sequence
  primer pENTR1A-4
agtcgactggatccggtaccgccaccatgaggaagcccaagaagaagcccaagaagcccaggtccagcgggggcgaggag

SEQ ID NO: 181 - DNA, 61 bp, Artificial Sequence
  primer pENTR1A-Flag-GFP
gtctagatatctcgagttacttgtcgtcgtcgtccttgtagtccctgtacagctcgtccat

SEQ ID NO: 182 - DNA, 54 bp, Artificial Sequence
  mCWSP-AD-BsestAF
acttactgttgctcccatggctttcgctgcagatgctgaacacaatccagtcgt

SEQ ID NO: 183 - DNA, 43 bp, Artificial Sequence
  BsestAR-HA
gtaatctggtacatcatatgggtattaattcgtattctggccc

SEQ ID NO: 184 - DNA, 90 bp, Artificial Sequence
  mCWSP-AD-PX12-20-BsestAF
acttactgttgctcccatggctttcgctgcagatagaaaacctggtaaaggtcctggtaaacctagatccgctgaacacaatccagtcgt

SEQ ID NO: 185 - protein, 181 aa, Bacillus subtilis
AEHNPVVMVHGIGGASFNFAGIKSYLVSQGWSRDKLYAVDFWDKTGTNYNNGPVLSRFVQKVLDETGAKKVDIVAHSMGGANTLYYIKNLDGGNKVANVVTLGGANRLTTGKALPGTDPNQKILYTSIYSSADMIVMNYLSRLDGARNVQIHGVGHIGLLYSSQVNSLIKEGLNGGGQNTN

SEQ ID NO: 186 - DNA, 543 bp, Bacillus subtilis
gctgaacacaatccagtcgttatggttcacggtattggaggggcatcattcaattttgcgggaattaagagctatctcgtatctcagggctggtcgcgggacaagctgtatgcagttgatttttgggacaagacaggcacaaattataacaatggaccggtattatcacgatttgtgcaaaaggttttagatgaaacgggtgcgaaaaaagtggatattgtcgctcacagcatggggggcgcgaacacactttactacataaaaaatctggacggcggaaataaagttgcaaacgtcgtgacgcttggcggcgcgaaccgtttgacgacaggcaaggcgcttccgggaacagatccaaatcaaaagattttatacacatccatttacagcagtgccgatatgattgtcatgaattacttatcaagattagatggtgctagaaacgttcaaatccatggcgttggacacatcggccttctgtacagcagccaagtcaacagcctgattaaagaagggctgaacggcgggggccagaatacgaat